European Patent Application EP 4 596 572 A1, published August 6, 2025. Title: A fusion protein that forms self-assembly comprising an intrinsically disordered peptide tag in which major amino acids are composed of charged and hydrophobic amino acids, and a method for purifying recombinant protein using the same. Applicant: CCRIPO Inc. Application KR. The sequence listing filed with the application follows.

SEQUENCE LISTING (40 sequences)

SEQ ID NO: 1 - protein, 6 aa, synthetic construct
  REGION 1..6: note = His6 tag_AA
HHHHHH

SEQ ID NO: 2 - protein, 18 aa, synthetic construct
  REGION 1..18: note = PSIAEH tag_AA
PSIAEHPSIAEHPSIAEH

SEQ ID NO: 3 - protein, 21 aa, synthetic construct
  REGION 1..21: note = PSIAHEK tag_AA
PSIAHEKPSIAHEKPSIAHEK

SEQ ID NO: 4 - protein, 30 aa, synthetic construct
  REGION 1..30: note = PSIHEKIHEK tag_AA
PSIHEKIHEKPSIHEKIHEKPSIHEKIHEK

SEQ ID NO: 5 - protein, 12 aa, synthetic construct
  REGION 1..12: note = PSIA tag_AA
PSIAPSIAPSIA

SEQ ID NO: 6 - protein, 28 aa, synthetic construct
  REGION 1..28: note = His6: PSIAEH clone_AA
MDPMHHHHHHPSIAEHPSIAEHPSIAEH

SEQ ID NO: 7 - protein, 31 aa, synthetic construct
  REGION 1..31: note = His6: PSIAHEK clone_AA
MDPMHHHHHHPSIAHEKPSIAHEKPSIAHEK

SEQ ID NO: 8 - protein, 40 aa, synthetic construct
  REGION 1..40: note = His6: PSIHEKIHEK clone_AA
MDPMHHHHHHPSIHEKIHEKPSIHEKIHEKPSIHEKIHEK

SEQ ID NO: 9 - protein, 22 aa, synthetic construct
  REGION 1..22: note = His6: PSIA clone_AA
MDPMHHHHHHPSIAPSIAPSIA

SEQ ID NO: 10 - protein, 22 aa, synthetic construct
  REGION 1..22: note = PSIAEH clone_AA
MDPMPSIAEHPSIAEHPSIAEH

SEQ ID NO: 11 - protein, 25 aa, synthetic construct
  REGION 1..25: note = PSIAHEK clone_AA
MDPMPSIAHEKPSIAHEKPSIAHEK

SEQ ID NO: 12 - protein, 34 aa, synthetic construct
  REGION 1..34: note = PSIHEKIHEK clone_AA
MDPMPSIHEKIHEKPSIHEKIHEKPSIHEKIHEK

SEQ ID NO: 13 - protein, 287 aa, synthetic construct
  REGION 1..287: note = His6:PSIAHEK:TEV protease clone_AA
MDPMHHHHHHPSIAHEKPSIAHEKPSIAHEKGTGSPPVPSTPPTPSPSCRSGESLFKGPRDYNPISSTICHLTNESDGHTTSLYGIGFGPFIITNKHLFRRNNGTLLVQSLHGVFKVKNTTTLQQHLIDGRDMIIIRMPKDFPPFPQKLKFREPQREERICLVTTNFQTKSMSSMVSDTSCTFPSSDGIFWKHWIQTKDGQCGSPLVSTRDGFIVGIHSASNFTNTNNYFTSVPKNFMELLTNQEAQQWVSGWRLNADSVLWGGHKVFMVKPEEPFQPVKEATQLMN

SEQ ID NO: 14 - protein, 220 aa, synthetic construct
  REGION 1..220: note = His6:PSIAEH:INF-a2 clone_AA
MDPMHHHHHHPSIAEHPSIAEHPSIAEHGTGSPPVPSTPPTPSPSCRSENLYFQGCDLPQTHSLGSRRTLMLLAQMRRISLFSCLKDRHDFGFPQEEFGNQFQKAETIPVLHEMIQQIFNLFSTKDSSAAWDETLLDKFYTELYQQLNDLEACVIQGVGVTETPLMKEDSILAVRKYFQRITLYLKEKKYSPCAWEVVRAEIMRSFSLSTNLQESLRSKE

SEQ ID NO: 15 - protein, 244 aa, synthetic construct
  REGION 1..244: note = His6:PSIHEKIHEK:rhG-CSF clone_AA
MDPMHHHHHHPSIHEKIHEKPSIHEKIHEKPSIHEKIHEKGTGSPPVPSTPPTPSPSCRSAAAENLYFQGTPLGPASSLPQSFLLKCLEQVRKIQGDGAALQEKLCATYKLCHPEELVLLGHSLGIPWAPLSSCPSQALQLAGCLSQLHSGLFLYQGLLQALEGISPELGPTLDTLQLDVADFATTIWQQMEELGMAPALQPTQGAMPAFASAFQRRAGGVLVASHLQSFLEVSYRVLRHLAQP

SEQ ID NO: 16 - protein, 296 aa, synthetic construct
  REGION 1..296: note = His6:PSIHEKIHEK:TEV protease clone_AA
MDPMHHHHHHPSIHEKIHEKPSIHEKIHEKPSIHEKIHEKGTGSPPVPSTPPTPSPSCRSGESLFKGPRDYNPISSTICHLTNESDGHTTSLYGIGFGPFIITNKHLFRRNNGTLLVQSLHGVFKVKNTTTLQQHLIDGRDMIIIRMPKDFPPFPQKLKFREPQREERICLVTTNFQTKSMSSMVSDTSCTFPSSDGIFWKHWIQTKDGQCGSPLVSTRDGFIVGIHSASNFTNTNNYFTSVPKNFMELLTNQEAQQWVSGWRLNADSVLWGGHKVFMVKPEEPFQPVKEATQLMN

SEQ ID NO: 17 - protein, 278 aa, synthetic construct
  REGION 1..278: note = His6:PSIA:TEV protease clone_AA
MDPMHHHHHHPSIAPSIAPSIAGTGSPPVPSTPPTPSPSCRSGESLFKGPRDYNPISSTICHLTNESDGHTTSLYGIGFGPFIITNKHLFRRNNGTLLVQSLHGVFKVKNTTTLQQHLIDGRDMIIIRMPKDFPPFPQKLKFREPQREERICLVTTNFQTKSMSSMVSDTSCTFPSSDGIFWKHWIQTKDGQCGSPLVSTRDGFIVGIHSASNFTNTNNYFTSVPKNFMELLTNQEAQQWVSGWRLNADSVLWGGHKVFMVKPEEPFQPVKEATQLMN

SEQ ID NO: 18 - protein, 232 aa, synthetic construct
  REGION 1..232: note = His6:PSIHEKIHEK:INF-a2 clone_AA
MDPMHHHHHHPSIHEKIHEKPSIHEKIHEKPSIHEKIHEKGTGSPPVPSTPPTPSPSCRSENLYFQGCDLPQTHSLGSRRTLMLLAQMRRISLFSCLKDRHDFGFPQEEFGNQFQKAETIPVLHEMIQQIFNLFSTKDSSAAWDETLLDKFYTELYQQLNDLEACVIQGVGVTETPLMKEDSILAVRKYFQRITLYLKEKKYSPCAWEVVRAEIMRSFSLSTNLQESLRSKE

SEQ ID NO: 19 - protein, 237 aa, synthetic construct
  REGION 1..237: note = GFP_AA
SKGEELFTGVVPILVELDGDVNGHKFSVSGEGEGDATYGKLTLKFICTTGKLPVPWPTLVTTFSYGVQCFSRYPDHMKRHDFFKSAMPEGYVQERTIFFKDDGNYKTRAEVKFEGDTLVNRIELKGIDFKEDGNILGHKLEYNYNSHNVYIMADKQKNGIKANFKTRHNIEDGGVQLADHYQQNTPIGDGPVLLPDNHYLSTQSALSKDPNEKRDHMVLLEFVTAAGITHGMDELYK

SEQ ID NO: 20 - protein, 16 aa, synthetic construct
  REGION 1..16: note = Hinge_AA
GSPPVPSTPPTPSPSC

SEQ ID NO: 21 - DNA, 18 bp, synthetic construct
  misc_feature 1..18: note = His6 tag_NT
  source 1..18: mol_type = other DNA
catcaccatcaccaccat

SEQ ID NO: 22 - DNA, 54 bp, synthetic construct
  misc_feature 1..54: note = PSIAEH tag_NT
  source 1..54: mol_type = other DNA
ccaagtattgctgagcatcctagcatagcagaacacccaagtatagcagagcat

SEQ ID NO: 23 - DNA, 63 bp, synthetic construct
  misc_feature 1..63: note = PSIAHEK tag_NT
  source 1..63: mol_type = other DNA
ccaagtattgctcatgaaaagcctagcatagcacacgagaagccaagtatagcacatgagaaa

SEQ ID NO: 24 - DNA, 90 bp, synthetic construct
  misc_feature 1..90: note = PSIHEKIHEK tag_NT
  source 1..90: mol_type = other DNA
ccaagtattcatgaaaagatccacgagaagcctagcatccacgagaagattcatgagaagccgagtatacacgaaaagattcacgagaag

SEQ ID NO: 25 - DNA, 36 bp, synthetic construct
  misc_feature 1..36: note = PSIA tag_NT
  source 1..36: mol_type = other DNA
ccaagtattgctcctagcatagcaccaagtatagca

SEQ ID NO: 26 - DNA, 84 bp, synthetic construct
  misc_feature 1..84: note = His6: PSIAEH clone_NT
  source 1..84: mol_type = other DNA
atggatccaatgcatcaccatcaccaccatccaagtattgctgagcatcctagcatagcagaacacccaagtatagcagagcat

SEQ ID NO: 27 - DNA, 93 bp, synthetic construct
  misc_feature 1..93: note = His6: PSIAHEK clone_NT
  source 1..93: mol_type = other DNA
atggatccaatgcatcaccatcaccaccatccaagtattgctcatgaaaagcctagcatagcacacgagaagccaagtatagcacatgagaaa

SEQ ID NO: 28 - DNA, 120 bp, synthetic construct
  misc_feature 1..120: note = His6: PSIHEKIHEK clone_NT
  source 1..120: mol_type = other DNA
atggatccaatgcatcaccatcaccaccatccaagtattcatgaaaagatccacgagaagcctagcatccacgagaagattcatgagaagccgagtatacacgaaaagattcacgagaag

SEQ ID NO: 29 - DNA, 66 bp, synthetic construct
  misc_feature 1..66: note = His6: PSIA clone_NT
  source 1..66: mol_type = other DNA
atggatccaatgcatcaccatcaccaccatccaagtattgctcctagcatagcaccaagtatagca

SEQ ID NO: 30 - DNA, 66 bp, synthetic construct
  misc_feature 1..66: note = PSIAEH clone_NT
  source 1..66: mol_type = other DNA
atggatccaatgccaagtattgctgagcatcctagcatagcagaacacccaagtatagcagagcat

SEQ ID NO: 31 - DNA, 75 bp, synthetic construct
  misc_feature 1..75: note = PSIAHEK clone_NT
  source 1..75: mol_type = other DNA
atggatccaatgccaagtattgctcatgaaaagcctagcatagcacacgagaagccaagtatagcacatgagaaa

SEQ ID NO: 32 - DNA, 102 bp, synthetic construct
  misc_feature 1..102: note = PSIHEKIHEK clone_NT
  source 1..102: mol_type = other DNA
atggatccaatgccaagtattcatgaaaagatccacgagaagcctagcatccacgagaagattcatgagaagccgagtatacacgaaaagattcacgagaag

SEQ ID NO: 33 - DNA, 864 bp, synthetic construct
  misc_feature 1..864: note = His6:PSIAHEK:TEV protease clone_NT
  source 1..864: mol_type = other DNA
atggatccaatgcatcaccatcaccaccatccaagtattgctcatgaaaagcctagcatagcacacgagaagccaagtatagcacatgagaaaggtaccggttctccaccagtaccaagcacacctccaactccgagtccgagttgtagatctggagaaagcttgtttaaggggccgcgtgattacaacccgatatcgagcaccatttgtcatttgacgaatgaatctgatgggcacacaacatcgttgtatggtattggatttggtcccttcatcattacaaacaagcacttgtttagaagaaataatggaacactgttggtccaatcactacatggtgtattcaaggtcaagaacaccacgactttgcaacaacacctcattgatgggagggacatgataattattcgcatgcctaaggatttcccaccatttcctcaaaagctgaaatttagagagccacaaagggaagagcgcatatgtcttgtgacaaccaacttccaaactaagagcatgtctagcatggtgtcagacactagttgcacattcccttcatctgatggcatattctggaagcattggattcaaaccaaggatgggcagtgtggcagtccattagtatcaactagagatgggttcattgttggtatacactcagcatcgaatttcaccaacacaaacaattatttcacaagcgtgccgaaaaacttcatggaattgttgacaaatcaggaggcgcagcagtgggttagtggttggcgattaaatgctgactcagtattgtgggggggccataaagttttcatggtgaaacctgaagagccttttcagccagttaaggaagcgactcaacttatgaattaa

SEQ ID NO: 34 - DNA, 663 bp, synthetic construct
  misc_feature 1..663: note = His6:PSIAEH:INF-a2 clone_NT
  source 1..663: mol_type = other DNA
atggatccaatgcatcaccatcaccaccatccaagtattgctgagcatcctagcatagcagaacacccaagtatagcagagcatggtaccggttctccaccagtaccaagcacacctccaactccgagtccgagttgtagatctgaaaacctgtattttcagggctgcgatctcccacaaacccactccttaggttctcgacgtactctaatgcttctcgctcagatgaggaggatttcacttttcagttgtttgaaggatcgtcacgacttcggatttccccaagaagagtttggaaaccaattccaaaaggctgagacaattccagttttgcacgaaatgattcaacaaatctttaatctgtttagcactaaggatagcagcgcagcatgggatgaaacactccttgataaattttatacagaattatatcagcaactgaatgaccttgaggcatgcgtcatacagggtgttggggtaacagagactcctctcatgaaagaagacagtattttagccgttcgtaaatattttcagcgtattactctttatcttaaagaaaaaaaatactccccttgcgcatgggaggttgtccgagcagaaattatgaggagcttctccctctctacaaatctgcaagagtctttgagaagtaaagaatga

SEQ ID NO: 35 - DNA, 735 bp, synthetic construct
  misc_feature 1..735: note = His6:PSIHEKIHEK:rhG-CSF clone_NT
  source 1..735: mol_type = other DNA
atggatccaatgcatcaccatcaccaccatccaagtattcatgaaaagatccacgagaagcctagcatccacgagaagattcatgagaagccgagtatacacgaaaagattcacgagaagggtaccggttctccaccagtaccaagcacacctccaactccgagtccgagttgtagatctgcggccgcagaaaacctgtattttcagggcacccccctgggccctgccagctccctgccccagagcttcctgctcaagtgcttagagcaagtgaggaagatccagggcgatggcgcagcgctccaggagaagctgtgtgccacctacaagctgtgccaccccgaggagctggtgctgctcggacactctctgggcatcccctgggctcccctgagcagctgccccagccaggccctacagctggcaggctgcttgagccaactccatagcggccttttcctctaccaggggctcctacaggccctggaagggatctcccccgagttgggtcccaccttggacacactacagctggacgtcgccgactttgccaccaccatctggcagcagatggaagaactgggaatggcccctgccctacagcccacccagggtgccatgccggccttcgcctctgctttccagcgccgggcaggaggggtcctagttgcctcccatctacagagcttcctggaggtgtcgtaccgcgttctacgccaccttgcccagccctga

SEQ ID NO: 36 - DNA, 891 bp, synthetic construct
  misc_feature 1..891: note = His6:PSIHEKIHEK:TEV protease clone_NT
  source 1..891: mol_type = other DNA
atggatccaatgcatcaccatcaccaccatccaagtattcatgaaaagatccacgagaagcctagcatccacgagaagattcatgagaagccgagtatacacgaaaagattcacgagaagggtaccggttctccaccagtaccaagcacacctccaactccgagtccgagttgtagatctggagaaagcttgtttaaggggccgcgtgattacaacccgatatcgagcaccatttgtcatttgacgaatgaatctgatgggcacacaacatcgttgtatggtattggatttggtcccttcatcattacaaacaagcacttgtttagaagaaataatggaacactgttggtccaatcactacatggtgtattcaaggtcaagaacaccacgactttgcaacaacacctcattgatgggagggacatgataattattcgcatgcctaaggatttcccaccatttcctcaaaagctgaaatttagagagccacaaagggaagagcgcatatgtcttgtgacaaccaacttccaaactaagagcatgtctagcatggtgtcagacactagttgcacattcccttcatctgatggcatattctggaagcattggattcaaaccaaggatgggcagtgtggcagtccattagtatcaactagagatgggttcattgttggtatacactcagcatcgaatttcaccaacacaaacaattatttcacaagcgtgccgaaaaacttcatggaattgttgacaaatcaggaggcgcagcagtgggttagtggttggcgattaaatgctgactcagtattgtgggggggccataaagttttcatggtgaaacctgaagagccttttcagccagttaaggaagcgactcaacttatgaattga

SEQ ID NO: 37 - DNA, 837 bp, synthetic construct
  misc_feature 1..837: note = His6:PSIA:TEV protease clone_NT
  source 1..837: mol_type = other DNA
atggatccaatgcatcaccatcaccaccatccaagtattgctcctagcatagcaccaagtatagcaggtaccggttctccaccagtaccaagcacacctccaactccgagtccgagttgtagatctggagaaagcttgtttaaggggccgcgtgattacaacccgatatcgagcaccatttgtcatttgacgaatgaatctgatgggcacacaacatcgttgtatggtattggatttggtcccttcatcattacaaacaagcacttgtttagaagaaataatggaacactgttggtccaatcactacatggtgtattcaaggtcaagaacaccacgactttgcaacaacacctcattgatgggagggacatgataattattcgcatgcctaaggatttcccaccatttcctcaaaagctgaaatttagagagccacaaagggaagagcgcatatgtcttgtgacaaccaacttccaaactaagagcatgtctagcatggtgtcagacactagttgcacattcccttcatctgatggcatattctggaagcattggattcaaaccaaggatgggcagtgtggcagtccattagtatcaactagagatgggttcattgttggtatacactcagcatcgaatttcaccaacacaaacaattatttcacaagcgtgccgaaaaacttcatggaattgttgacaaatcaggaggcgcagcagtgggttagtggttggcgattaaatgctgactcagtattgtgggggggccataaagttttcatggtgaaacctgaagagccttttcagccagttaaggaagcgactcaacttatgaattga

SEQ ID NO: 38 - DNA, 699 bp, synthetic construct
  misc_feature 1..699: note = His6:PSIHEKIHEK:INF-a2 clone_NT
  source 1..699: mol_type = other DNA
atggatccaatgcatcaccatcaccaccatccaagtattcatgaaaagatccacgagaagcctagcatccacgagaagattcatgagaagccgagtatacacgaaaagattcacgagaagggtaccggttctccaccagtaccaagcacacctccaactccgagtccgagttgtagatctgaaaacctgtattttcagggctgcgatctcccacaaacccactccttaggttctcgacgtactctaatgcttctcgctcagatgaggaggatttcacttttcagttgtttgaaggatcgtcacgacttcggatttccccaagaagagtttggaaaccaattccaaaaggctgagacaattccagttttgcacgaaatgattcaacaaatctttaatctgtttagcactaaggatagcagcgcagcatgggatgaaacactccttgataaattttatacagaattatatcagcaactgaatgaccttgaggcatgcgtcatacagggtgttggggtaacagagactcctctcatgaaagaagacagtattttagccgttcgtaaatattttcagcgtattactctttatcttaaagaaaaaaaatactccccttgcgcatgggaggttgtccgagcagaaattatgaggagcttctccctctctacaaatctgcaagagtctttgagaagtaaagaatga

SEQ ID NO: 39 - DNA, 714 bp, synthetic construct
  misc_feature 1..714: note = GFP_NT
  source 1..714: mol_type = other DNA
agtaaaggagaggagttgtttactggtgttgtcccgattttagttgaacttgacggtgatgttaatgggcacaagttctctgtcagtggagaaggggaaggcgatgcaacatatggtaagctcacgttgaagtttatttgcactactggaaaactccctgttccgtggccaacacttgtgactacgttttcttacggtgttcagtgtttttcaagataccctgatcatatgaagcggcacgatttctttaagagcgcgatgcctgagggatacgtgcaggaaagaaccatcttcttcaaggacgacggtaattataagacacgtgctgaagttaagttcgagggagacaccttggtgaatcgaatagaacttaaaggaatcgattttaaggaagatggaaacattctcggccacaagttggagtacaactacaactcacataacgtatacataatggcagataagcaaaagaacggcatcaaggcaaacttcaagaccaggcacaatatcgaggatgggggtgtgcaactagctgatcattatcagcaaaatactccaattggtgatggacctgtcctcttaccagataatcattatctgtccacgcaatctgccctgtcgaaggaccccaacgaaaagagagaccatatggtgcttcttgagttcgtaacagctgctgggattacacatggtatggacgagctatataagtga

SEQ ID NO: 40 - DNA, 48 bp, synthetic construct
  misc_feature 1..48: note = Hinge_NT
  source 1..48: mol_type = other DNA
ggttctccaccagtaccaagcacacctccaactccgagtccgagttgt